European Patent Application EP 4 585 700 A2, published July 16, 2025. Title: Zwiększenie specyficzności identyfikacji jednonukleotydowych polimorfizmów genetycznych w układach izotermalnych poprzez zastosowanie oligonukleotydów z powtarzajacymi się modyfikacjami typu LNA. Applicant: Instytut Biotechnologii i Medycyny Molekularnej. Application PL P.447279, filed December 23, 2023. The sequence listing filed with the application follows.

SEQUENCE LISTING (14 sequences)

SEQ ID NO: 1 - DNA, 43 bp, Homo sapiens
  source 1..43: mol_type = other DNA
acactatgctacggcaatatgcacggagaatctatgaacactc

SEQ ID NO: 2 - DNA, 43 bp, Homo sapiens
  source 1..43: mol_type = genomic DNA
cacagaaccatgcccgagagaacccacataagtctttccaagt

SEQ ID NO: 3 - DNA, 43 bp, Homo sapiens
  source 1..43: mol_type = genomic DNA
caaagaaccatgcccgagagaacccacataagtctttccaagt

SEQ ID NO: 4 - DNA, 19 bp, Homo sapiens
  source 1..19: mol_type = other DNA
tgtcattcctggcatgatg

SEQ ID NO: 5 - DNA, 18 bp, Homo sapiens
  source 1..18: mol_type = other DNA
cactgacaagccaccatt

SEQ ID NO: 6 - DNA, 20 bp, Homo sapiens
  source 1..20: mol_type = other DNA
acaggacagtcctaggcatt

SEQ ID NO: 7 - DNA, 21 bp, Homo sapiens
  source 1..21: mol_type = other DNA
tcaagggctcatgtttctcaa

SEQ ID NO: 8 - DNA, 535 bp, Homo sapiens
  source 1..535: mol_type = other DNA
tcatgtatttggaatgaggatattagcagtatttatttcatggtatggttctcagaactcagtgtgtttatatacatgaagagcttaggaaagtatttggttagtcagcactatataagttgtcattcctggcatgatgtttagtagtattatcactgtgtatagtcatgacttatcttcaattttaagcaatctttaattgatacggagaatctatgaacactccaaatgcctaggactgtcctgtgcatattgccgtagcatagtgtgaaatttcctgaacttttcaggcanagaaccatgcccgagagaaatagaagaataaaaaagtactcaagggctcatgtttctcaaacttggaaagacttatgtgggggaggaatggtggcttgtcagtgctatatacagagttagagaataaagacagcatgtttttacagaatatcacatttactaggaaaatgtaagtaacataacattaggtaatattgaatcatccagaaatatcatagaataaaggtaaagttgacataat

SEQ ID NO: 9 - DNA, 43 bp, Homo sapiens; identical to SEQ ID NO: 2
  source 1..43: mol_type = other DNA

SEQ ID NO: 10 - DNA, 43 bp, Homo sapiens; identical to SEQ ID NO: 3
  source 1..43: mol_type = other DNA

SEQ ID NO: 11 - DNA, 43 bp, Homo sapiens; identical to SEQ ID NO: 2
  source 1..43: mol_type = other DNA

SEQ ID NO: 12 - DNA, 43 bp, Homo sapiens; identical to SEQ ID NO: 3
  source 1..43: mol_type = other DNA

SEQ ID NO: 13 - DNA, 43 bp, Homo sapiens; identical to SEQ ID NO: 2
  source 1..43: mol_type = other DNA

SEQ ID NO: 14 - DNA, 43 bp, Homo sapiens; identical to SEQ ID NO: 3
  source 1..43: mol_type = other DNA